European Patent Application EP 4 123 020 A1, published January 25, 2023. Title: New biological nitrification-inhibiting bacteriophages and their use. Applicant: FERTINAGRO BIOTECH, S.L. The sequence listing filed with the application follows.

SEQUENCE LISTING (1 sequence)

SEQ ID NO: 1 - DNA, 42088 bp, Viruses
  SEQ ID NO:1
agattgatttccacgtaggtaaatgtgtgagtgtggtgactcaatatgtactcccacggtatagagatacaggagtttcatttgagataatgaggcgagcaaggagggaatgtaaagcacaaggagtgggtatgcttgcttggtctcatagggtcagggattttgaatacaaaacggtttataggagtgtgggatgaaaaagattttcaaggctgttgtaggtggaggcggcgggggtggaccatcaaaggaggaagccgccgcagcagaaagagcagcggcagaggctaacctgagggctcaacaagcagcacaggcgttgcaggaaaactttcgtgctgatctgagtacagacaatatcgcccagatcgctccgggtggtgaagctaatgctgcagggatggatgatgatttcaccccgcaaagaaaacgcaatagggtaggcggattgtctactcagttaggtatagggggtgacacatggctgtagatcaacgtcttcagagtacatgggctgccctggttgcagcagcgaattcctataacaaaaataagagcactcgttacctaactgatgtgaggggtaacaagattctcgatcctatacaaccagcgcgatcctacgctgatatgcagagagagaagctagggatggtccctgaggttggggatttcttaggcttgaacttggatccggatggtgtgagtggtaaccgtgatacgggagttcagaaagcattgagtgattatagcgccgcccagagaacagtagctcatgaacagcagggtttgattccaagccctgccccacaaccatcagaatcacgagggcagcttagagttgatctggatacttctccggtacaaactaaagactcagtaatgtaccgtaatgctggggaaggggaagagggtactataggtgaggctagtagaccgaataaacgtaagcctggtctttcctctaatctggggattaacctctaggaggagatatggctaccaataaggggctatttgagaaataccgggacacctatgtgttagatagggcaacacaatatgcaacgtggacactccccgccttaatggccgatctccagcaaacctccaacggaacacgtactgttctgcaaactgacttccaagaaattggagcactccttaccaacaatctatcctctaaactagctaggatattattccctacccaatattctttcttcaaggccgatgcaagtggtgaactggcagaggtaatgcgggaacaagcaggtgatgagagcaatttccgcgctaccttctccaaattggaacgagaagccaataagaacctcttcatgaattccgggtattcttcactgatactcatgcttaaacatttgatagtcactggtaacgcggtgatctatcgtgatagcaaacgtaaaaccattactgtctatggtcttcaatccttctctatcaaacgagatggtagaggggatgtagtggactgtattatccgtgaatatactctggttagttccctccccgaatccatcattaaagaacttaagaaaaaagacttagggagattcaatgaccctaactctgtagtagaggtttatactcggatcagaagagagtacgttaaagacgagcctaccatggcggttactactgaggtaggggatatatcagtaggtgaggagggtaggtacccggttgagttatgtccttatatcttccctacgtggtctcttatccatggggagagttatggacgtgggcttgtaggtgacttcgctggagggtttgctaagctctcagaactatctcgatctggtgctctttactcagtagagactttacgggttatcaatctggtggggcctgcctcaggtacggacgtagatgcaatagccaacgcggaatctggtcagtgggtgcgtggagaccctaaggagataagtgcctacgagtcagggcaggccaataagctccagatagtaggtgcacagatcaacgaattaattcagcgcctctctgtggctttcatgtacacagggggaggggcgattagagaaagtgagagaacgacggctacggaagtagctatgttagctcaggaagctgagttaaccttaggcggggtctatagcgccttaagtgcatccactcaggttccacttgcttacttacttatgttggaggtatcagcggatgcgttaccgggtatcatttcgggagaattacttcctgatgttacagtgggaatccctgccctcggtagatcgggggatgtgcagaatttactactggccgcccaggagatagcaggaatagctcctatagtccaacttgatagacgacttaacccagctaagatagtggatgtgattctatccggaaggagtgttgatccagcatcaattatgtatacccctgaggaacagagggctaatgatgaggcagccgctgctgctcagcaggcacaggctcaattacaacaggctgacgtgttagccaacacaacagcgttaactggaggttaagaatggctgatgataatataaatggtgtacaacctgcgcctacagggacgcccactccacctgccggtcatggtggagcacagtttgcaggacagagcccaggatgggtagctaacccaggtggaatggggaatacaggaacctttactcaggagcaggttaaggctatggtggctgatgcagtggctaaggctactcaaggattacctaaagcccctcctacctcctttaattctaacggaacccccaacactagtccccacgcagctaatcatgaaccattagtggactttggaggaagtcttaactccttcgatgtcaatagcattgatgatcctgtactgcgttccatggctactatgttcaagtctagtgtaccagatatggatttggatagagccttagctaacgctatcagctatggtgatcctaacctgatagatatcgcttacattaaagataaagcgggtcagaatgctcctcatttaattaatcttgccgctggcattgtcaatacgatcaatgctcaatcagaggccatggagcaatctgtttatcaggaggttggcggtaggcaggtatgggatgcctcagtagccgtgtttaatcgatctgcatcacctgagatcaaggctacggtggctactatgttggatagtggaaaagctaacctgattaaagctggggctaggatggttgctgagtttggtaagagtagcgggatgatccctaaagacggcttccgacttgatccggtatcagccccctacgccaatcaagggttgagtaaagctcagtttcaacaagagatactcaaactggatagcaatgctccagattatgctgataagtacaatgccttgattcaacggagagtagtaggtaagcgtttaaatcttaattaaggagtgttatgttcacattgattcttttgattcttgtagtgttctttgccaatgtcatcgttgacactgcccgccttgatggtggtggaacaagtagattctgggtagtgctgttctcagaatgcaaggtatgggctgtagcctactgggctgtagtggatagcaagattcaaaatttacttaataaatcaatctaaggagtgagtaatgcctacaccgtataatacaactatgagtcgtgcgcattgggctggtaccgatgcggatatggatatccatctggaggcatacgaaggacagatcgaaggttccttccgtgttgaaagtatgttccgctccagtggcctgactcaattcaaacaagtacgtcaacaaagcaatacatggcgcggtgatcggattggtggcgcggtggttaaaggtcgtaaggccggtgatagtctggacagtacccgtattgtgaatgagaaagtactcgtcactgtagagtacaccagctatactcgtactccaattgactaccaagacgattggacggcacctgacttcaaggctcagtacagtgctgagcagggtagtgcccatgccaaagtgttcgatcaaagccacattatccaacttatcaaagctggtacttggcttgctcctgcctctctgaaagcgtctggcgcttttaacgatggtattcgtaagaccatgactggctacgctgctgctctagccctaaataccgaagcgggtaatgagactgctgcggggcttctggtcaagaatcacaaggaagcactggcgaccttcgtcaagcgtgacctaggtggtagcctggctgagtttgtcactctagttgatccggatactttcaacgtgttgttggatcataagaaactgatgaacgttgattggcaaggtagtagtcagggcgtaggtaacaacttcgctatgagacgtattgcatggatgaatggtattcgtgttatcgagactcctcgtttccctacttctacgatcactgatcatccgctgggagttaacttccatctcgatgctacggaggctaaagctcgttgtgtcatcttccatcctcgtaaagctctggtaacagtggaggctcaaccgatgaaaagccgtttctgggacgatgaggcgaatttcaccaacgtactggatagctatacgatgtacaccgtaggtctcctgcgtggtgatgcagtagcagttctggcaacagactaaccttagaatggctaggattagattctaaggggtttaatgaggaagggtatataagactatacctttcctctatttagttccttaaattgattcctagagctttctggaggtattatgcaattactgtttgcagttaattcgatactccctaaattaggggagcgtcctgtaacgtcattggaagtaaagcacccaacactggctatcgtattaccagtgattgagatgcagcgtaggtcattattacagcgtggctggtggtttaatgagtttaaatacacagcttaccctaacctagatggggagatattcctaggatcagatttcttgtctttcattcccaaggtgccattagcggcagcagtcaggggtgagagattgtataacccaactaccttatcctataagtttgatgagcctgtagagggtaaagtaattcaggatgtagagtttgaattccttcctgatacagcagccagggcagtactatacttctctctatcagaggtttacgtgaccgatcttgatatgacgaatgaggtacaagagtggaaaggattagcagcagaggcatggaatggattacttaccgaacacttgaggcaaatgcggtattccacccaaggtatgcggacatggaatagaataacatcacagatgaggagctagtatggctgcctatgcttcagcgtataaagccttcctgcaaggcgtatctcaacagattccttctgagaggctatcggggcaggctacggcacaacataacatgctatccgatcctgtcacaggagttagacgtagattaggtgtccagttcaagaagcaatttcaatggactggtattagcaaaagtaacttacaggcatggtttacggatgtaggtggtagtcccattcacatactggttaataccaccgcagggacaattaagatactgaattcctcccttgtagaggaggccaccctgggccctgtagcgtatctacaggccacaaatagacgttctatcagaggtgcctcagttggacaggaattcttcctctgcaatactgagaaggatccgagtgtatctactgctgctgtaggtcttaacccggatagaacaggatacttctatgtggtagccggtgccttcagtagagcatacaatgttaccatcacgtatggtggtactaccttcaccgtgacctataccacacccaatggagcttcccctggggatgcggcattatccactcccgagtacatagccgaacagttagtgaatggtataacgagcactgcgccttccctcggtatacagagagatgggccttatgtctatgtggtcaatgcagcaggtactttgaggattaacacctcagcagggactcagtacatgcaggttagtaagatgtcctccgctagaactgttggagacttgccagccagactgccttctaacgctgatggttataatgtaagggtaggcgtgggcggtacgtaccagtattacaggtataatgcctctactactgaatgggtagaagtaggatcgtatgcaggccctagcggtataaccaatgctccaatcagtatatactggaacgggtccgcatgggcgttgaacacatccgctttcaatgggagaccatcgggagatgatgactcgaaccctaagcacgaatggatgacttacgggatatcaggtatgggtacctaccaaggtagacttgttatactatccggtcctatggtgtctatgagtgccagtaataagccgcgtgacttcttccgtaccacagtcacatcagtagttagctctgacccaatcgaggtaggtagtagtaccaacagctcagcagcttacgagtggtgtattccattccagaaggatttagttgttttcagtaacagttaccaggctgttgtcccatcagggaatgcagcagtgactccctctacagcagtcgtagtccctacctcaagtttctcggctgatacaacttgctctccgatatcgataggtagaacacttctgtacgctaagcctaggtcggataacttctttggtatcctagagatgttacctagtagctacacagatagtcaatatacctcaacagatacaacacctcatctcccacggtatatgcccgggaggtgtagtcatgcagccgcctccagtgtggctaacatagcggcctttgtccctactggggatgattcatcagcgatcatccatgagtaccattgggatgcagataacaaggtgcagcaggcatggcacacatggtcattcccctacccagtagcagcactttatttctcccaggacgtgatgagtatttgctttgctcagaatgattacctggtaataggtgctattgatgtgcgggcgggtaacgtggctgtagatggtactagaaggccattcttagatatctatgggaatatcagtatagtagctggagtcgggaccattccagcttggatgctagccttcgaccctgatatcggagataagataagattaatccaggctaccggtaatctggctggggaggctatcgggtttgaggtgtcaggtaatacaataactactgtacccagcttccaggatgggacagctgtgcttggattaccctatatgtcgtccatagcgattcctgggcctatagatagagattacaatggtaaccctatctacacaggtaaagtaacgctacagcgcattataatcggtactagaggctcttctgagtttgatatatccgtgactgatgatagatcggggatggatgaggggacagtacctaccctgtacatgagtagtaaagaattagagttaggtagaggactgtacggagatatagccagttcggtagtaccatgcaggacagacgcccgcaccacggtagtagagatgtcaacagataagacaggggagataaacataacctctatcgagtacatagcaagagcacaccaccctataaggagaagataatggcggctatgttagggatgatggcggtgcaggctggcttgtccttcttaggaggacaatctgcgaaggcgcaggccaaggctcagttacgcactcagcaaatagcagatagcaaagaaatagtgagagataggctgcaagccagtatacgtaatgcttacgctactgccttaggacaagttcaattagctctgaataagaaacagacagcacagcagatgtcgagtgtcagagctgggggagtaagtgccttaggggatgcttccctgatgtctgcctattcaggcaccatgggggcttcagtagatgcagtatctagtgatataatgcagcgtagtaatgaggcgctgactcagttgcaggagaactatgacgcctctttacatgactacaacagaagcttggatgctatggtagtcaatactgagctaagcacgcctcagcagagggagtataaatacatggggcctagtactatggataacctattaggtgcagtaactgggacagctttatccttcgccggtaactacgccaataagaagatgaagctagaattgcaggaagttgtaaagaaaggctcttcaattagcagtatattaggattctaggagattctatgagatcgtatcgccctgtagacttcggaattagggatacccgccaagttcagggcgggcaggttacagcaggatcgagaggagcaggtgcccctgttatggcaggggacgctgggtggagggggaggttcctcagccaactatctgatcaggtaggtagacatgtaatagacaccttcaacactgaaatagagagacggtatttagatggacaatcccgagccctcatggatgagagtgaagaggagattcagggagacccattaaccaaagactgggaagtggctgggttcagagatgcgaagggtaagttagctctggccgatatggatgtaaagttcagggaggatttaccagagctaaccaagaaacccgcagaagaggttaaatcttatctgtctagtagacgggcagagatgacccctttactctcttctatgactagggaggctaaagcctctatcatggggcagatgtacctgcgggatagggcacatattaaaacgtggcaatcagcacatcaggcatacatccttgagcagaagcggtctgctatagctacccagaattcagtgtcccttcaaggcatggtggcagcacgatccgcttaccttaatggggatttgtcggcggacgcatacgccgcaacggtagagagcacggcgggctctttgattggtagtatcaatatggatgagtcactaccaaccaatataaagaatgccttaacagaggaagctattcagtactctcttgagaatgacaatccggcactgtatgagttccttagggataacactgtacctgattctaatggtactcagtacaatgtactggctaagcttcctcaggaatcccagatcaagcttagtaaagcataccgtggttcctatgaccgtaataaggtagcccgtaacgtaggttatcaggcagaagtagccaaccttaagaaccaattgagtcttggtacctatggaggaacctatgaggagttacaagactttctcggtaggatgaccattaaccaagcagttagtcaagggcaggcagtcaagatgcttgaggactacttgagtatgagtagcaataactcacagaatgcggctataatggaagcagtaacctctggtgataccaacaggctacatatgttgggagttactgaggataatgcttggaaggtacagcaagaggcatggagcaagcagggagttcctttacagtcccaggtaggtatgtccattctcatcggggagaagtccccttccgggtataagcaggcaggtatcctctctaacagttccattgataaggttcgtctggcttctgaagctggaggtgatgagcggggagaagtgaacgagacggatagagaggtgttccgtatctacaatgagggagtgtaccaagcagccagagagaatcagcaggtcaagctaactgctatgcttgcagggctatctcctgataatgcctcctacatggctgatatagccgagagaatgaatcagggggagtccctgggacgtgcccagttcaatgccaataaggcgtacaatgagagtaaagcattctcccccagtaaaagggctgggctggcacaatctacgcggaaagcagttagggatcaggttaactctgatctgaccccccgtaactggcttgaatcagcatggggtgagttaaagagtgtaatccccggcaccaatgctgctgtggatcaagggttgagagcagagtccagtatggatcaattctggggagattcagaagccactcagtacatacaatataatatcaatcaggatgttatacaagcggctgacaggatacttcaggagaaaccctaccttcctacagatgctgcgattaacgctgctaaggcagataccctgcgcagaactgtacgcgggaataacatgatgtatgttatccctgctgatgctgatgtacagaaactttatggtgttggacctgatgctagagccaagatcggggctgctatgcaggagatgttctctactaagtctcccgataataagttctatgtgtggcataacggccctaatgtcatggctatggaattcaagcctgatgggaccgcagtaggaacggagtttgtcatatctcctacagaagttagagcaggtatacgtaggatggatgagaggatcaggaaatctaatgatgaggtatacggagcgggtaaagtattccctatcaaggaaggaggttccatccgtgtaaatggggagaatggtgtaggtgtatctgagaaaactatgttcagattcagaaagaacctgatacagagtgaaggagttagaagctcatcctatagagactcatctaagaagaagattccaaccaatggagtagggttcagcgttaagtctaagcattacaaagcaggtaccatgactcctgaagagattcagaaaggattaatagctgaatcagatgagaagatgaagtacgctcttcctgtagcccagaggtacaacctaaatgaggcggggctgttattcgtggctgaggttaactaccagtcaggtccgggtgcatggactctggaggatagagcagcgaaacatcatgcagtactggctgctattcaatcaggagatagtaaagctgctatggaagctttgaataagctcccttcttatagagaagctggggatagtagaaagagacactatgcggcattagtgattgaagcatcaaagcgttaaacttacgagaatgcgattctaggggccattgtattgcaggtaggcaatactagccccgagtacataagcacccctagaatcgcatcctagtcggtttgagaggtattctttaggagaaggtaatgatagaatctatagaccaaagtaaacggcctactatttatgtaacaggtaagcctagagtggatgttcctgaattaccctcccctaatgatcaggtagaaggagggagagtagaccccggccctaccccatcagccagggttatagatgagaccctggatgcctcgcagtcaattcagaacagagctaaaggcatagccgagcaggatagagaggatgttactgtatgggatagcataggagcttctgttgcggtatgggatggaacaaggatagttgataggttccaaagacctacctttggggtaaccacgcctgtagagaatgttactgagtatttagagaatgcgggagtagtactaaattcagacgaaagggattacgtcttatccatgtctgatagtcaggaatcactggactatgctatcaactatgttaaggatcaacagagagcacgtagtatatcgggagagaatcctaaaacagcattactcacagcctttcttgatcctgcttatcttgtacttcctgctggtatacgagtgggtagagtagcctccgcggttactatgggtggagtcactacgggcataggtcacgcagtggagggtgtggtatcggatgaggagttattgcgtaggatacttattaactctggtctaggtgcggcctttggtaagatgaaaggaactggtcctagtgctactatgatcaccaagaaagctcctgatgacatatctaacaaggtggttaacgaagcggtggtcccatcagctcctcccgaaggatggtccaagaaggtaggagatgctatatcattaaacatccataaagaaattagtgggtttggggatgtaggtaaacgagtagcagatactatattcgataacaactctaacttaggtattaactcagttgagagttacagagaagcggctaagagtactctgacctcataccaaataaagtttgaagataccatgcgtgaggctatggcggagcgtggtgtaggtacaggtacaatgattaatcctttcaaatcccgtaatgctatggcagttcagcgggagatagaggaggaggtagcccgggagatggcaagacgggaatctctaacctttcaaggtatcacagactttactaaccctaacatctcaaagaaggtgagtgagatagcggattctctggccgagcttcacgctaaagcacttgaattgagtaaggcagcaggtgtagtaggcactgataagatagctaagaatcctggctatatccgtagagtgtgggatagtactaagatacaggctaagatagatgacctcataaaagatgggcttactgagcgtaaggctaggaatagtcttagtaaagtaattgccgctgctatgctgaaggttaatccacagataggcgctaagatagcattacgcacaggtaaatcaatcattgaccgtaccttgaagaaaggatacttcgaagatgtcctcagcaatgaggggctgtacggggcaggctgggctgagagtatgcgggatgctatgaagtcagcaggtgtacctaaagacaagatagatgaagctttagaggcattgtctggatcagtaggggaaacaggtaagtcctcattcctgaagaatagaatcgatatggatgcggatgtgtctgtcacgttgggcaataagccagtaacgtacatggatttggtagacacaaggattaccaccaatgtggataactacttacagcatgtgagcactgatataggatttgcatcagcggggattaaagatcagaatgctatccttaagatgaggactgatttactgcacagtatagccgatcctaagaagagagagaaagccgccgagttatttgatgaaactatcaagagtctcaaggggctgccagcaggtgggaatgttcctgagatgcttaggggattgaacagttataatagactgataaccttgggtggatcaggtctatggcagttaacagagtacagtacagcagcagttaagtttggtatggctaacaccataaagtacgccgtgaaggaaatacccggtataaggaaactgcttcatcccaacacgatggatgctggaacattagcgagagtcttgtcagatcaaagctcacaaagtatcaggatgcgtccgtatctagctaagtttgatgatggctttgctatgagtactacctccggcttccaactggcagcacaggccgctaaccataatctccctctgttcaatggaatgaagtatatccataagcaccaggcgaggattgcaggtaacctcatgcaggagttagtagaatcagcggtaaaagggaactccaaatctcttactcaattatcgaagtacgggatgactgatgagattatggcgggtatcagggaagaagtcaagaagcatggtatgcaggttgataagtgggcagatgctaattggcttaaggctaatactgtgttctccaagatgatggacgaggctgtgttacgaggtagaatgggggataagccatcctggatactgttctcccctgtaggtaagaccttgttcatgtacaaagactttgtaatgactgcccataataagttactggcaggatcattgaagagggacggagctagtgcagtaggtatgatgttattataccagatgcccttaacctatatggctgtatctgctagagcggctatggcaggtgagcagaaatcaaatgatgaactaataacggatgcagtgagttacttagggacgttgggtctactgtctgaaatagccggtgtggctactggtggttctggttcatggttctcctcagtaggcatccctcttaacagagcaagtaacttagctagatcaatacctgaagctatgtcaggagatgtatctaagactggaggaacactcatgcagatgatacctctcatatcagcccttcccttcatgtcaggcgtagctaagagagtaagagaaatggaagattgattatagactctattaaatgagattctaggggttattgtgccttagtgtacactaacccctcaactaacctataaaccctctagaatcaattcctagaggcttctggaggtatttatggcattaagcaacatgacgatagtttcggatgggaatctggagtttgtatccatctcattcaactatctggacagatcagaaataaacgtttacttcgactcaataccaaatagcacatgggcatgggtaggagatactaatcagattaagtttactccaaaggttcccaatggggtaactgttcttatagctaggatgactgatgcatcttatttacgacacgtcttctctgaaggagcagcatttactgctcaaactctggatgaggatttgaggcaggttctccatattgtgcaggaagcgaaggaaactaatctgtctggtgacttctattcagatattgatatgcatggtttccagataaataacctgggtactgctacagatgacaatcaagccgtatcactgggtcaataccgagctgacgtgctaggagcaggtgtagcgcgagatgaagcggaagggtatagggaccagactctagcttatcgtaatcaagcagagggtttcaagaacactgctcagtcgtcagctactaccgctaccactcaagcaggaatagcaacgactcaagctggtatagccacaactcaggcagggaacgcttcaacttcagccagcaatgctctcagttatcgtaacactaccttgacctacagaaatgcagcggaggggttccgtaatgaggcagaggggtttagggatgacgctcaacaggctgtgatagatgcctctgatgcatcaaggctaacagcgggaacagtaaccacaggtagtcccggaactagtgcggctgctaccataacaggccctgctggtgcccaagtactcaatctcacattgcctagaggtaatgagggatatagttactatgcatggtctacggcgggaaacctcactaatatttccagtatatctggcatgaaagtaggtgattatgtagttaatacctctggggctacccgcactatgctgggggtttccactgcggtgggaggtgtagtaaggagttcaggggctactacagggacagcagcaggtagtatactaggccccgcagtacccctggttcaggtgaaaggaacgagtactacctcagcaatgagtcagaatgccgttactaatgagttaacggaggggactactaccactctaggggcagcagctttcagggaagtctatctatcaggagcagccccgagtcctggtgaagtaatggcagcttccccagttactatagagcttaattataatggctcaggcaatagaactagcaatatagatttccactcacgagatggtacaaattacgatgcgaggataataaagaactccggagctagtggaacctttgatcttatcgccactaacggctcaatagctaacattattaatctacaatctgacacccatacagttgactttaactacagtagtctcacaggtgtgcgcattataagatatccggtaggggcaggtagcgctggtgaggtacgtgttcttcataatggccccccatttggtactggttactatacctgttattatgggggtgttttaagtggcagtataacagcagcatctagttcttctgtctctttcaatactacttcagattaccgacttaaagagcaagtacttcctatggtaggcgctcttgatagaatcatggcagctaaaccagtaacctataaatggaaatctgatggcagtgctggagaaggttttattgcacatgagttagctgaagtagttccgctagctgttactggtgagaaggatgctgtagatgaagatggtaaacctaagcaccaacaggttgattactcgcggctaacgcccctacttactaaaggaatacaggagttaactcttagtattcagagtctacagtccactatcaaagagttagaagatagaataactgatttggagaataactatgagtgagttagacgacctccacctgttaaagaaacttttaatcaagtcccttactacaaggttcaaggaggatctagaaaatgaatctggcttcctccctacagatgcagccactatgaatgcagccattgcattactgaagcataacaacattacttcagaccctaaagatgcggatgaccttaatgaactacgcgatcgattacgggaatcgcagaaggctcgtagaagcgcaggaagcaacgtagtagacttagctgagggtaacctagctaaactgagagaaaagctctagaatcgaatcctagagcttcttgtaggtgttgttactaaagagggtctaggatggatttacaaacaagattcaaacacgctgatttaatagcagagacttaccaatactttcctgacttcgcagcagatgcacttaggttcatagggtttaccataacccctatgcagttagatatatcagactacatagcctatggtcctaagttcaggatgatcatggcagggaggggagaggctaaatccacccttgcctatatctactccatatggagattgatccagaggccatctaccatcgtgttcgtagttaccagtaaggagaaactgtctctgcaggtagccaccggtatgaaacagttattgttccagtgggatatattagagtacatgagacctgataagaatgcaggagatagggtggctactgagtcatttgatattcactatgcccttaagggggttaataagtccccttctgtctccattggtagtatcactggtggtatcactggtaaccgtgctgacttcctattatcggatgatatagaaagtgaagctaactcagataccgcagctaagagggatactatcaaggcagccactcaggaatacacctcaatttgtagggatggggatattatgtacataggtactccccagaccaaagattctgtctataatggacttcctaatcgcggtgtggatatacgtatctggccttctagggtgcctacctttgaagaagaggagcgttatttcggtaggctggctccctatatccagcagatgatgctgaaccctgataacaggaaaggttatggattgactggtacccaaggtaaacctaccgatccagttatgctgtctgagcagaagcttatcgaaacctacgtggatcaaggtccagagaagttccagttgcagttcatgttggatagtactctcagtgatgagatacgaatgcagcttaagctaagcgacctggtggtggctaacttcggatgtgatgtgttacctgaggtggttcagtaccagagtagtcctgctaaccaggttcctctagggagtgacttccctgtacctttagccgctatgtactacgcctctagtctacagtgcgcgatggttaaacctaccgaggtagtgatgtgtattgatccggctatgtccggctctgacgctttaggattcgctgtaggtacctctgtggggccttacatccatatcctcgatgctggtggattgatgggcggatacaacgataagaatgaggaagagctgaagcagatcatgatccggaataaggttactcgtatagtagtagagagtaatatgggacatggtctattcgagatcaacctaagagcggtactacaagctgatgacagagtgtctcatctagcaggatgtgttgaaggcaagtacgctacaggtcagaaagagaagcgtatcatagagagtctggtgtcacctatgcagaggcatagagtaatagttcaccagcaagtattcgattctgataggaagtacctgaagcaacactcatccgataagaggacagagtatagtctatggtaccagttaagctcaatcactaccgacagaggatccctcaaccatgacgacgtattagaggcggtgagtatggtagtaagggagcttaaatttgatctggacatagaagaggatgcagcagcagaggctaggaaacaagcagcaataagggagtatttagcgaatcctatggggtacaagaataccaagaaaacccgaggtagggggactttatctaaacttaggatggttaactaagaggaaatcatgaaagagtattcgagcactaacgcctacctggggggcatagcggcagttgtagggagcatgacattacaagactgggggattatagtgggtatactggttggggtagggactttcttccttaactggtattataaagctaaagaattggaattaaaggagaaatcccctagtgttgttattcataaggagtaacaatggttaatcgatctaaactaattgctggaaccggcatcatgtctatggtggcagtgttatcactatcacctatgggactagatactattaaacagaatgagggattacgtactactcagtattatgatcaagccggggtagcaactatctgctacgggagcaccggtaccggattaaagacagccactgtagagaagtgtaatgaactccttaagagacacactgacgatgcagatagagtcttgaagaagtacatcaaggtggaactaactcaggaacagtatgatgccctccatgacttcgttcaccagtatggggaaggtaagttcaaggcttctaccctcctgaagaaaattaactccggtgattgtaaaggggctgtagaccaattccctagatggagactggttaacggtgagtttaataaaggcgtctacaataggagtctaaggaatgctgctaagtttagttcgggctgtattcactggaagcaaaattaagtggtatatcctcggggctctaggatgcgttttaagcgtgtttctcactgtagggtatataaaggtactcaagagtgatataaaagccctagaatcgaatcgtagtgctttgcaggaacattcccagtctttagagaaccagctagaggtttataaagatgcagtagagaatctagggaaggttaacaagaagaatagaggggagttagattccaagctatccacactacagggggcaataagtgaagaaagacgactggctgatggcactggagctaaccctatcggggatagttctgcttgtcctagtgagtgccttaacaggctgcgcaggatcaccaaagaggccaataaacagtttagataaggtaatggtaccctcagcctgcttagagacgcctaaagcgatcctagagccttctaggggcattattgatgagtacatcgatttagtagtgcaatacacggacttagccatattgaagaatcagtgtagagaattcttacttaaggggaaataatttggctagcgtgaatagacttactagggatgatgtgaggcgggattttgtgtataaccctgatgagggtactttgatatggaacaccttctcaggatcatctacgccgggggatacagcagggtggcttgataagtatggttatgtgagggttaggtatcggagaaagatttactttgctgcccaactaatctacctgcacatgagagggaatataccggatgggatggagatcgatcacattaatagaatccctaacgataaccggtgggataacttgcgtttagtaactaggtctcagaacaaacgcaatagagtattgtgcaataaaactggactcactggagttagtaaagcgtctcctaacaggtggacatcatgcattaaactgggagatcgccgtagaaggttggggctattcactacccctaaacaagcgcataacgcgtatttattcgcagcatctttaacttaacaggagaaagtaaatgactattgcttcaggtaccgccaccaatgaagaattggtaactctttacaaagagactgctatcttagaaaccatgctccgtcaattcaatgatgggtcagctaaggataaggataaacccggtagattcacccccgctcaaatggatgctcagatcactaaagtgagtagcgccattaccgcagttaacgctggggcttgatgactaattaatccaatccagagtaataccctcccctgcctaaggtggggggggggaggggaatgatatgagggaataacaatgatattaatgggaacatctaacactactaatcacttcacaacaccatcttacacattaccggatacaccagaggtgacaattctattaggtgggcggatagagggtcatccatcaggagcaacacaaggactgatagcatggggtggggatgtttctttccgagcatttgttgctggttcaggtaatttagtaatcaccaggcccaccggtactgactttaacaacgctggggtagccgcgtccacaataggcaaccctacagaatttatattaggtatccatataaacagggataccccgtctttagggtatgtaacctttgctctactgggacagcctatatttaaatctgccagtgtcaatttaggcagtcctgtggaactagtgaaccttgttctggggaatgtagttcctctggatcgcccgcttcggctcggtagcggaatcaatttcttatctgtagtcgcaggagcgttcccagttgatcttattcagcaggtagtaaacggggagacacaacttgagacggaacctaacgtggtatctaccttccacttcatccaatcaacacagcctgtattcgttgatgcgtctatgaataccatacaagctgtgggaagctcctgggggccggactttgaccctgagcttaaggcatctccttctccagttaactcaactgtatcgtatttaaccagagcattaacgaagtgcctctctgccaccagctattaccgtcagggggatgctcgtaacaagcagaaacctggtccatttacccctagtgagattaataagctgatcaatgatgtcaaatcagccagttcatctctaacaggtatattcctctaaacaacaccacgagagcccctcagaattgactaagatttgattctaggggctttcctccttcagtaatacctttctataccttatctagtaatacctcctctatggagattctaaggcttcctagagctatatgtcttatgtagcccttctgtagcctttctgtagcctctaattcgtagcaatcgaaaataatatataattccgaggggcctccccgccccgccccactcttctttcccccgtaggccccctattgattatctgagaagatgatcagataagtgctacatctcatccattatgtagcactccttattattacaccttattatagtagttctattattactcctagttactcctaggtgcactactcttcagtattactcttcattactatgctgcttgttgcttgtttgactttgtgtgggggaggtggcttttttggtgaggtttaacgagtttttttagtgagttctccctctctctctctcttgcttggtgagatttaatctgcttcttagtgagacttcttttggtgagggtgaaggtgatacttcataggcttttggtgggagttgtgagtctcttttgtgagtctcttttgtgagtctcttttgtgagtctcttttgtgagtctccttttactcatggagctctaatcgattctatcatcgtagaatgtctttgatcgggtagtactaacggtttttgtgtttttgattcgaacggtacctttccttccgttgtttattaatatatcaaagaatgtaacttcaaatttatttttgttacagtactcaactaagtatatgtatataatagtgaatccgaaaattcccgctttaagtgaagtaagttaaagaaacaagttgacaagttgataataaaggtatagaatacaccacataaactaagatcaacagggaggagatgagatgatctgggttatagctgaatggatttctgaagtgattcaaagtatattaaacagaatgagaggtaaataatgagctacgatgatgcagtgagggaagctagtagagttaagtcctactatccttataggatcgttggtgtagtaagcaaagatggtgtagtatgggaaacattatcaggtaagaccatgagtagattcaacagtcgattaaagaaaggttatcaggtagtattacttgaacgtgttctgtaggaggttaaatcgtgtactcgcaagtaaaagtcaagtataaatggttagcagtggtcaaagagaattgctgtctaggtagtagaggaacagtaataggtaggagtaataattatggatacctgttcaggaggtacaccaataacaaatacccggtgcatattatgtacactactaatctaaacccagagatacgggaagtactaagagagatagacttgcctcctaaatatgattaaagaaaactgttgacagggagttaataagagtataatatacatccatcaatcgagacaaaacttaaggagattaaaatgcatacatacactgatacccagaaagagatcataaacaacgtcaaaagcagacaagcggatattgattcctccacttgggcaggaggggatgcttttcacagctgcaggattttcctggaatgggcggaagcacatgctggagaaatctcgccagaagcagctagggagttcttctcccctctcgatcaccatgatcggctcgatgctgatctgtgggaactcaggggatattttctctcagggaagaagccatactacttataaatagatgaggagatattatgatctgggttattgcgcgatacatcaggaagtggatagaggatatcttaaaaggtagtaaataaagcttgacagcgtactcacaagcaggtatactaaacacagtcgtaaacactttaggagattgaaatggaactaacagtaaatataacttacttccctgtggagaagaagtacggggcatcattgtggttaggtgataagctggtagatataggttacaatctgtgcgatactaaacggaaggccatgaaaatggggggattgctcaagaacaattacatcaacaaggaaagggggagaataaaatgagtctttatacaacactccagaaacgaggatttccggagaaggaggctagccatatagcaacacaaatggcgaaccgatttggggagaagtttatcgaacttgatccagtgtgggttatgcatgaactggatgaggaattagttaatgacttaaaggaagaggatagagaggtatattggttcgaggtacacgaggagaagtattttgacggaggtatacgggtaccttactgtatacttatgtatgacatggctaaattaaggggtgacaatgacgtgtagcttcaatcacattgacaatatagtaggtaagatgcatgattttttattatggtctgaggacatcagtgcagaggagtggaagcagcatagtgatatagacttcatcgaagccttacgggtatacgcggatgaggtagaattctggctgggtgagtagaggagattataatgattaacaggtctaaagatagactagccctattccggaacagggccggggtagtgtctcccggaatacatggactggaggtagtgctgtatagtgagatagataattaccgctgtacccgcaagtcaattaatgccatatttccctatgatcctggtgatgaggtacttggtagacagtaccgggcagctaagaggcacctagataaattgtcggatgttaaataagatttgacaccttgaatcaatcctgtataatagaaccatcaattaacgcatcgagaaggggaaataaaatgagagaattagacttagatgaattgaatgaatctttgtatgaattgcaacaaaatttagttgaattacaattggagagagttagcacccaagagaagattgattcatttgacgcatctgaatatatatcctatgaagaatatgatgacttcatcaatgaaatacacggtgcaacagtggatattgccggatcagtatttgatcccgcccgcgtcttaagggtacttgataggagtgcatataatcttggatataatgattattgtgcaaattataacattgaggacatcccagaatacagggtacttacagaaagactaaatgaagtagagtctgaaatgaggtatattgaaaatcagattgaagaattacaagaaggggttgacagagcatcacaagaagggtaatatgcagcacatcatatagcaactggttaccgcgagacgaaagagctgcgaggtagggtttagtaaagggtaagtggcgattacctaccagtgtcgaaaacatcctagaccattggtcagataagtaggcagttagatgatagtagtaatcaaggcggttgaatcggggaaagattggaaggatacctgaatgaaacagtttgaagaagtaaaagacggtcgcagcatttactggccgtatggtttaacagtacgaatggatagaataacagccggtatagctctcagaagatatagtgagactctgccggtagatacagaagtagatttatgtgtaaagggcgaagaagagacagaagtacatttcctcagaatgcccttgacaagtagcaagaagtagggtagcatgcaccaaatcagctagagattaactactagccccggcctgaaacctagcgggtaaaactaggacagaaccatagccgatggtttcctcgggcttgataaatgaggaagaagtttagggtaactagacagcgtgagataggatgctctactcacaagcggaatcggctcactaagtggaggatgcagttagttctgatccgtggaaacttagttggtagggagacatattagccttacccgatcatagggcttatatatataagtaactagatagtatacccggtgctcagtcgagcggtatgccgggtataccagtgtagttattctaaacaataaaccaggaggaaattatgaacgcttatcaacaattaaacgattatcttgtagatgtaggtgtagaggtgaagatagaaaggaatactacgttcgaacgaaaagacttccccgaagggagtagacattacaatgtaacagtgtctaaccaatcgggagattccttcctgcgagtgtactcgcaggggcctgctattgaagacgagccaagtatattggccgtgttgcactcattagtgttagattacgattgtggggaactgtccttcgatgatttctgttccgacctgggatataatgcggatagtagggaggattataaactatggcgctccgcgaaattgataaacgtggagatgtttaatatcctaggaaacgatgtgatagatcgtatccgtgatatactatcggattactaagatgagcatcagatcgacgtgctataagatatcgaaagtactcccaatagtgggaagtatggctgtcgggtggatggtgtacggtgactttcagccggtaccagccgcccctttgacagataaacaagcatggcctaatgtgacgagttatgagtcatgcgacgtatatccaacggtgaggtacactggcccggtatgtgaggattgtaaggatggtgtacccgtaagtgatggtggattacatagccctcacaatgataatctgtataagtacctacctaagaatggctcaggaatcgattatattggcccttcctgcggtttaattgcggagggtaagggtaacactgtgcccgagcctgaaaccttcttaaacgtaattctaggaggttttattataatatgtataaggaggagatatgttggtaatcaacaaacatagaggcagaataataaacccctgcgattccctaaaagggcatttatggcgggggataagcgaaactacttatcaatgtgcgagatgcggagagtgtgcaaatcacgaagatttcgcggtagaaggggagagtggaggggatcatgaaaaggactagcggacgagccgtcgtgaatgaccgggatgaatggtgcaagaaagatatggttacatgggcgacagagatatgtctgcttagcctggtaatagcactgtgggttaatgttcttgtttacttttgctctggggtatagggatgtctaattacggatacttagcagtagatgaggatggtactattgtactgttccgagataaacctgacatcgctttcctttctccctattataaaggtggtaaatactggtcaagagtaggtgcggactacctaatagtaactgttaatctgaataacgtcagaagattacgagtaaactctaagactcaatacggccctatatatcatatagagttggactataacggtcactattacgtatcattgaataagatcaaggatacgactcctcatgtagccccattctttgttgcgttaccgacaggtctaaagatacgtaaagggattttgaaaggaaagtatcaccgatgagagatcatgattggactgtactgtcggtattcttcgggaggtaatatggataacaatttttggcggcatgtcgaaattgatgccgaaggcagagtagtgttgtataaggatcaccatggaggcggtgacacggaatcaatctgcctccctttggatttccccttaactaggaagttaaggttgactactaataaacagcatcagagaaaagtagtactcaggcagacaacctcgggtgactactttatggaatatgagacgaggtccggaagggtgtcatatagcggtctacaaaaagctccttgtgtattccccctacctgagcctattgtagcacgaggtaaatttttccgagaggggcttagacatgcgagataatgattgggctgttcttttgttggtgggtgtggctgtcttaatactgtacatgcaacctaaacaggcgcgcgcatccgctagcggtatctgcaaggcatatggcgatggcgcggcagttgtgcatcaaacaattagtgaggggtacagtcccagaggatcacttgaggcactagcgcaggtacttcaggataccgcgccgctgaatagcaatactctagctatattacgtggagcacaagagcgagtagctcaggatagcagcatagacaaagatgctcctgctgaaatggttcaggatgtattcttccaggactgtatcaaactggtgtatatattagagatggatcgggtgggaaaatgaaatcgaaaagagaagaatttaagatggccctaataatggaaatgatagttgcctgtgacttgagctgctcccggcgagaggttaaacctcttaccccgaaagaatgccgggagcttattggtctcttagacggatatcttgatagagtcactgcggcaagagtaggggtaggttgagtataacctggcccatagctaaccagcgtacttagaatgagaattattaatattactggagattatgaatgtggttaattggatcgattatgctaagcaagctaattccggggggcgtcccgtccgtttcggtcattgtggaaactctggcaggaatgccgtggcgtacaacaatccacggggctacagcgctaagtgctatagctgtggctggaaggactacaaggcaaagaaactctacatctctaaaggggcggcgggtgaggatcacaaaccgggggtacgagttagccctgtaccagtagataaactaatcccagagtttagtgaggtggtgtggaagtacaccctacagtatggtatgaccccggaagaggctggagtaaaggggatttatagggataggatcatagtggaatgtggtgatgtacagaaaggaaggcgagtaccctttctggacaaattcggaataggtgctaaatgggtgacctatactgacggtgtggctatggtaggtagtggggatatattagtagccgtggaagatatgctctctatgtacaaagtccacttagccctgccagatatatcagttatatgtctactcggaaccagttttaaatcactctaccgtacacacttagagggggttgtagaaatttgctggatgctagatggtgacggagctggagcgcggggggtggtaaaaggtatgcgggaactggcgccttgggttagaaagcagagggtaataatgctgccctcaggaagagacccaaaagatttacatattaaagaaatacaggagcttttccatgatcgatagtatgttactagtgtctatgagattacgagacacgtactaccgtttgaaggacaagataccggaggatttagtcagcagtgacaccgtagggatccttaagtggtatggtgctttcctaaaagcatttccagatagtgatagcgtggaatatgaggcattctccgagttcatacgcttacgcctgagtagaatgccggataaaatggagttgatgttaaacctctggaaagagataaacatagaacctacttattacctacctccaggggatttagagttactgatagaagatgtatggctagctggtagggtaggtatgatttcctcccagtaccaagccggggaggagattgacctaaaagcggagttgacagccgcccttaatgagcataattccgaggggaatgatgctgaatttgacggaaccagtatcacggacatccttaatgagtttagcgaggagggagggtttactttcggattctgtagaatgctacgggatagcctgtacccagtaaccccggggaatttaatcatggtagccgctcgtgtcaatcaaggaaaaacttctctactctgtcggatactggctgactggtcacagcaggttgagaaggtatacgggtgcaagcgtcccatcatgtatcttaacaacgagtcagcggtatctcgtatcaaaggtaggatgtatcaggcagctcttagagccactataccagagctgcaaaatataggtgacgaggaagagctggataatgcgttcagattagcaactaacgattgtgaattcctcttcaaaaatattcatggccgggacgtatccaaggtggagtccctcgttaagcagtacgagccaggtattctacttatagacatgccagctaacttgaaattatctggtaagtttcacaatacggttgatgcggtagagcacatatggcaatcaatacgtgagtggtcagtactgtataatactgtggtgataggtactgcccagatcagtattgagggtgatgatatgctgttccccccactatcatcggtcaaagatagtaaaggtgcggtgcagggtgctctggacttgcaaattaatatggggtatgtgtcatccatgccgggactcagggggctgggggttgtgaaatctaaacgtatccgaccgggggtgggggtgatgcaggctgaagtatggtttaataacgataattgtacttttaacgacggagaataaaatgatacacactattaaagatgtagttaaatgggcggaggatcgcaacctcttaaacggctctactcgtaaggatcagatggttaagttagtagaagagataggcgagctagcttccggaatcgttaaatgcagggaggaggtagttctggactctatcggagatgctttggtggttctcattatcattgcagaacaatccggtaccagtatagaagaatgtctcggattagcgtggaacgggataaaagatcgcaaaggtaaaatggtggatggaatcttcattaaggagggagatcaatgaagaaatacctagcccttctcaagaaagttctggatgagggggaataccgggagggtagaactaatgtgggctacttgtccatattcggagagtcccttgatttcgatctgaaaaacggtaaattaccacttaccactaccaagaaactccacttaccttctatcatccacgagttactatggatgatcagtggggatactaatactaagtatctaaatgataacggtattactatctgggacgaatgggcagataattccggggggctagggcctatttatggggcacagtggagaaaatgggggggtgcccttaatcaccctggggtggatcagttaaagggggtaattaaggaaatcaaagagagccctaactcacgcaggctgttagtatcagcttggaatgtggatgagttaagtaatatggctttacctccgtgtcacgttatgttccagttttacgtgcagagaggtgagcttatgtgccagatgtaccagcgaagcgctgatatatttcttgggcttccatttaatatagcttcatatgcgctactaacccatatggtagctaaggtaactgggttagaggcaggtgctcttagggtagttataggagatgctcatctttatgttaaccatattaatcaggctagggaacagctaagtagacatgtgagcccacattgtccatggattaaaatacatggggagcacatcagtattgattcaattaaatacgacgatataacggtatctgggtattatccacatccagctatacccggcaaggtagctgtgtaaggggaattttatggatatagagagccaatgggtagtggataatatgtacatggtggatagagtcatacgtagacacttccctagcctgtatggggatattcttgacgaagccagggccgtaggtacggccgccatgtgggagcatagatcgacttacatagaggggaagggatgtagtgaagtgacttggttacaagatcgtattaaatgggcaataaacagatggctaccttatgacctttacgggttcagccaatccgtgtattacagattaagagaggaagaatccattccagattacattcactacgatcaaatggaaggccccgagggggatgataattggtatcttgacactgtagtcaaagaggatagagacccattaaaagtgttactggataaagagaggttggagttgttcaacgcagggttatctcttctaggacatttagagaggcgcgccttaatggggtatgcatttgatgctaagacatataaggaactagcacgggagttgaacaacaccgaagtaaatatgcagacatcagcacaaagagggagaaataaacttaagaaatttatacaggaggtgtacacgtaatggatgagtcaatagtgttcatcgattttgagactcagtctcacgagaagtacgggcataagtcttccccccataacccggataactttattgtagcggcggggtgggcttacggtaaggagggaccagtagagggggagtactattccgatgctggaggggtaactctaccattccttgataaccctagagtgaaaatgctcgtagcgcataatgcgccttttgatgcagggtggcttttatcccgacaccgctcccgattcatagagtttatccgtcggggtgggaggatatactgcactcaactggtggagtacctattgagtaatcaacaggatacatacccatctctggatgaagtggcaccaaagtatggtgggactcataaggtagatgcggttaaactactttgggagcaaggtgtactaacaagtgaaattgagcgggagttacttttcaccaagtacttaataggccctgagggtgatattgtgaacctaaggaaagtcttttatggacagatggaggagatcaaagagcgggatatgtggcagggtatactccgcaggatggatgcattactctttaatgtctttgctatggactcaggattgcacatagataaagatacagcgactcaaatgcattctgaaggggtagataaggtaaaggaattagaagcgattctggagcgatctagaggtattcccgaggaggttgggttcaaggtaacttccagatatcatgtttcagcgtggttattcggtggccccataacctacaaaacacgtgaacaggttatggccgatgaaggtaagccagtttacatagggtgcaacggataccaattcactgatgggttcttcattgaggagcacgacctagataattacaaaggggacttgtctaaacttgaggaagagcacggagagttaatccggtacaagtcgggtattaagaaagggctggctaaagtatttagaggtaagtctaaggaggtaaaaacacgatgggtggataaagtctaccaatgcaagggtgtgatagacctcagtaagctgcctggtgatttcgtggatagattcactgaggaacacacaggtaagcagaacttatctgatggaaccccggtgtatagtacatccgagaaagcaatagatagcctctctaagcaaccaggtgttccggaggaagccttaactatccttagggtaatgcaggaattgtttacctataacaagatattagggacttactacctgacagaagaaaaaggtagaacaagcggaatgcttcagtacatgacagactacaatgtggttcatcatagccttaacgctacttcaacagtaaccacgcggatgtcgagtacgaaaccgaatctgcaagtactccctcagaaaggagacgacttccccggtagaactaagaagctgttctccacccggtttgatgatccggtatgggtagactgggcagtgtctaattccataattccgaggggcgttgcggatgagctcccctttatccgtgagaaatatggtagagcaggagccatggtagcagtggacttcagcgctatcgagattgtggtaatggctatgctcagccgggatagtgcattgttaaaggcactgaaggaaggtactgatatgcactccctcagagtaagcaaaaatcacaacataccttacgaagaggtagtggaagctgttaacaatcacgaccacccgaagcacatggaaatgaaaaggcttaggacaaatatcaagcagccctcattcctttatgcctatggcggaactgctcaaggtatggtataccagctaggggttactatggaattcgcggagaagttcattaagacagagaaagcactgttccctgagcttgaagattatttcgagagggtgattgaagaagtggaatcatcttcctcccttcaccgtgagatggatgagaatggggtgtggagagtgttcggtagagggtaccagactatgccgtgcggcactaggttcgagtggcgacagtggcctaaaacggtatggcagaatgggcgtaaatcaaccaccatgcagtaccgaatacctgagatccgtaattattccagtcagggtacagcagccctcatcatgcaaattgctgtaggcatggtgatgagattggttactcataataaagagtgggatgggaaagtgttcctagtcaatcaagtacatgatgaatgtgttctcgattgcacgatggacgtagccgaagaagtagcaaggaaggtgcagcaagtaatggagtcagtaggtacagtgctggagaagttaggctatactgtgggattggaattcccagcagtacctgagataggtagtactttatgggataagtgtggaatcaactaagatttgattttaggaggtttaactgttatcttatagggtaagaagtacttagactataaagtttcttaaatcgcatcctagagccttctaggggcatttatataggagtagttatgtcattagatcgattgaagaaagccgcagatcaattcgtagaagaaacagcgcaggatttcacagaagcccaagctggtgcagctcaactgattcctgaaggatatgcctttgcccgtctagtagaatacatagagctgggaaaacacgctggggagtaccaaggtaagccacgtccccctgctctaatgttcaagctggggtttgccttgttcccaagtggggaggataccgaaggttatagttatgaggacggctctccaaaaatcatccgtaccttcgatattaacctgtctctcactgagaaaagcaaggctttcaaactattcaaaaagatgaacttcaaagggatacacaagcacttcgctcagatgataggagaacccttcctcttgaatgtggtgcatgttgacaaagcgagtggagggggtaaagcagcacgaattgatctggaagggttcctccctcccatcgatgtagtaacacgtaagccacacccgatacctaaagcacctgataacgtatacaagatgttcctatgggatcggcctaccaaagaggattgggactctctgtttgtggaaggtaagtgggataacggggacagtaaaaacttcatacaagagaagatactcgaagcatccgactttgaaggttccccactccatcaattacttgagggtgggaataaaaagaaagtacataaatcggtaactgagacaacagtcccggatatcccccaatatgacccatatgaagatgatattgatgatattatcccgttctgattatggatagattatcccggcttaaaggtatctccacagagctagataatcaatttgcggtagcctcttcgggggttaccgtactgatcgatggggatatcatagcgtataatgtcacagcaaatgtatctaagttgactacagccatacgaagatttcagcaggaagtactcaaggctatattcctaacaaaggcacagagggctatcgttcaccttacctcaagctctggggacaagaataaacgaaagctcatagttgctgatttaccttaccagagcaacagagctgggaaggataagcctccgctactagaagcgcttagagtaagtatgagtaaagaaaacaactggctagatatgttcgagtgttatttatgggaggacatagaagctgacgatgcccttatgattgatgctcataggctcaaggataaggggattatgtatagcgcggataaagacttaaggcagacaccgtacccttactatgagataaagacaggtaaactattccctgctctggatggcataggatgggttgatctaaggtatacagagaggagcaatggggtcggtaagctgacaggacatggggaattattcttatggactcagatgcttgccggggatactgtagacaacgttaggggactcaggaaagcctacgggaagaacatcggtgatacccgagcagtggaagagatgcgaggtataacagatcgagaggagatgatacataaggttacgcatctgtatgccactatcggtcagaacccaatacctgaactatggatgctgtatctgctacaagcaccagacaagacggctattgattacctgttggaacagcccgtttcccctgacgtgaggaagtggattaataaacttttaaaggaggttaaatggttaaagtagaagattaccgtaatgaatttaaaaccttaataagtaaactaccttttgaactcgatatacaaataattaactaccaactggtagggagtaccagtcataacggtgagggtggtgattacgatgttgtggtgttggtagccgaccttaatgagatggtaaatgggcttacattactaggatgggataatgaatcagatggggttgatgccaactatcctgtctctttcatcagtatgcgtaaagggaattttaatctaatactaacagtaaatggtgagttcttccatcgtatgaaaaactcagctgaggtaataagaaagatccagagtatattcggaagattggatagagcagatgtatgtgacatttactcaataattctgtatgggcatgcagtagatgaataaactacctcgcagcatgatgaagtcctggagcacacggcaactcaaagttgttcagggtggactgtgtgcagtgtgtaagaaacctatcgataccacaatcaagggggagggggtagtcgatcatgatcacattaccggggagataaggggagtgttacaccgttcgtgtaactccgctttaggtaaggtggatcatgctgtccgttgttggggaagcaaaggaggtacctatgaggatataattaactggcttaagaatatgctggaatactatgctcaacctggatgtggtctcatttacccttaccatctaaccccggaagagaaaaagcaggctgatttactccgtaggcgtagcaacagagcatccgccagagcgaaacagatactgaagaaggagactacatgagcgattggaaagaaaaggcgcttgatttagcctacgctggtatggtctggagcactatctcagaacaagtgggagaaccaaatactacggtgtataactatctcagggaagcattggggcctgcctacctgttccgtgagtctataaagccggaggataactcagccatcctaaatattcctgatttacacttcccttaccatcatggagattcgttcgatttcctacaggcggtcaaggaaaagtacaaacctactaggatagtgtgcctgggggatatggaggacatgcacgcgatgagttatcatgagcatgatcctgatttactcagtgctggttctgagctggaggaaacaagggagttgatccagcgtctgtatagtatgttcccaaggatggatatattagaaagtaatcatggttctctgacatggcgtaaggccaaaacccacggtataccccgggcttacatacgtgattataacgacgttctacgggttgggcctggctgggggtggcattacgacttgaccattaaactacctgatgggtcacccgtttattaccaccacggtaaatcggtcagtgtgttaagactatcccagcagatgggtatgtcagcagttcaaggacattaccatgagttattctcaattaactactggggtaatcctaatgggttgatgtggggattgcagagtgggtgcttaattgacttcagaagctacgcattcgcttatgcacgggttaatgttaagagacccgtgcttggatgcagcttgattattaactctcacccggtattagtgcctatggtgctggatagcggtggcagatggataggagaattatcatgacggtttcaattgaaacaatacatcaaagtgagtactgcaccatagcagtagccaggtttcaccctaggggaggtggattaggtaacgaattcgacgcagtatgcactctaatgatagagggaaccagttgtaaaataatagggttactcagcaaatctaccttcaaaataacccacataatgtcactatctaaggcattgcgatctcttggggtagagcgcgctttccttagacgtaacataacagagcctttcagagaattccacttaccagaatggaggttacattgagtaaagacgtactaccacgcaaagatgataaagggaaactcgactatacactactggatgatatgcccaatgctgtccgagcagtagtagaggtcatgcaatgggccaccacagagaagagcaacccttacgatagaggctccttcctttacgtacaccctaccaggtaccttgctgccatgcatagacactattgggctaccacagtggatcgtagagcagtagatgaggagagtcagaagctccatttagcacacatggcggtcagtgctatgatggccttagaaatgtatatgagaggggtagactgatgcagtttaatacacgcgaattcattgagttggcggaaagctcagcagaatgtctggagtatgttaagtcaggggagttcggccaagaacctgcccatgtcctggatgatctgattgtagaccttcaactatgccttacctgtacagaacaagcgagacataccatgcatgatatcctggacgtacttagacaaaaacgagaggaagtataatggaattccagaaaccgcagcagaatgattatgaatggttactggacaagatcaccatctgtatggagacaggtaattactcagcggccaaaactatcctaactgaaatgaatgaggatatccctctcgaagttaaagcagttaagcagagcattctaagagactacggagtcaaactttagtagtcccccaagcccctaggattcggttctaggggcttaaatacctctaggtatacaaaggtactaacggtatatcaaatcctcgtaatcttgatcctagtgagttttaaaatatggatagaaataaacaactggaatgggagagaagtactgaccttgaagctaaggcagaagcattacaaagattgaagagtgattcagagaagggtaaaactaacctacccagagccagagctatgttagggacaattttaccagatgtggagaggtatctgtcagaatcccttgacgtacgaacccatggtacaggggctaggtaccgggagtgggtaaggcagttaccagtggctgtagcctctgtaatagcaatccaacaatgtattcgtttactgagcaacaggaagcacttatctttccatagtgcgcagcacttgtgtagggaagtggggaaagagtatgtattagaagcacgtattcgtatggcgtcgaaggtatcccctatctctatgaaactggtttacaagcacataaaagatcagttggttagagacccacacagaatacggaagatgttcaagaataccatttctcgggtattcgatggagaattgaattattctatgtccgggatagcacatgcccagatagggaaattcggtatagatgcttgttggaaagccgggttgatagatatgcatcatatgaaatctaagcggggattcaaggtgatgtatcagttagtcccggaagtatacgagttcctagcagggtataatgatgaggatatctcgaagatagtgaaccctgattccggagttatgttatgcccaccagatagatggacttgcaacacggatggaggatacctgacataccaccgtaaaactagacgaccattattatcctctgatagtttaccgcaggggacagagagagaggctagagaagcggttgtattcgaaaaaatgcctaaggttttcaacgcggttaactacctccagtcaactccatttactatccacactccgactaaggaaggaatattgaaactgttttcagaaggagggggagttatgggggttcccaggaagcatcctccgtcaccccctccatttccgttcgaggatggattcgacataaaacaagccccgaaagagataataaaaaccttcgagcggtggaaagcctccaaaaagcgattctacaggcaggaggcagaatggaaagctaagatactagaggtggggcaattgttgcgtaatctcaattctagtgccttgcaggggcattccaggatatggtttcctacgtacctagattccagaggcagggtctactaccggggggtgattaatcctcagggatcagacatggctaaggcagtgatccactttgcagataagcgtccattagggtaccgtggattatactggttgaaggttggtatagccaatgcttacggatatgataaggtacgttttgatcaaagggctaaatggacagatgagaactggggaaagatagagcgtagtctggacaccccgtgggatcatccagaggtatggggaagtagcccttggtgtatgttctccttgtgctgggaattgagggaagcataccgatcaggaaatccggaaaagtacgagactggttgtgtagtacatatggacgccacctgtagcggtctggctcactactctgcattactgcttgatccagtaggggggcagtatactaatctgatagacatgggtactgacagtaagcaagatatttatgctaaggttgcctcagtagccattcaactagttgagcaggatttgttgagtgatgatccggaaatcaaagcgatggcggagtgggtaataaaaacagggattccaagagccgtagccaagagaccagttatggtgaaagtttacagtgctaccctgcatagtgcttctaattatgtatgggatgcttatgaaaacgaggtattcccgacaacaggtgaggaatggcctattcatttacacgtgccgaagtcaacgttttacatcgcagagaaattgttcttagggatcaagggtgcagttcctgccgctcactatgctatggagtggttgagtgaacagatgattaaaaatcgatctggtagagttaggtggacttctccctccgggtttatagtacatcacgattaccgactatacaaccagaaacgggttaaattgaatgcggctggggtaaccgctgtgatattcagggaggatacagacgagcagaataaacgctctatggcttcttccattgcccctaacttcattcactctatggatgcaagccacctagtcatgacagctaaccagatggagagagagaagttacctatgatagggattcacgactcgtttggtactcatccctcctgtgtggatagtatgcacaggataataagagatgagttcattaagatatacaagggtactaactggttatcctcatgggggctagaggtcaccggtatggagtgccctttaattagagggagccttgatatagataattgtaaagactcagaatttatgttttgttaaggtaagggaatttgaggttacatacttaggaaaggtagccaaaaattagagtttaatttgaagttacattcttagaacagatagccaagtttctgcattgactttacaaggtgcagcttcagcgacacagtgagacctcagggtgaagtgaagggtaactaacaattactcttcaccctaggaaaactactgaagagctaagatatactaaagtatataaatataattactatcgactctctctagagtataaaaagggggtagggggccttatatatatggtgagtaaaattaggattataagtaattgatttatatagagcgctaagtaggttttaagggggtttgctcagagagaataaccccacactttagtcaactatttgaagttacattcttagaggaggtagcaaaaatggatgaaatcaaattcagcgctgatcagttcagatggttaaggaagatgttccctaaccagatatggggccctggtactccccacgtgactatggtgtactataacggacagcaatcagtaattgaagcgattaaaaggcatactcatgggattcaagcgattcagggaataccggaggagtgaagggggagccctagtccacactcagttctatgctaacgcttgggaggagttcgttgagttacaatctcaacccaaagaggtatacgtagctaacgtcattgagtacctccaatccctgaaccgggtagagatctacgggtatatgcacggtagtcctattgggggagcggtactcacaaccgagattgatttccacgtaggtaaatgtgtgagtgtggtgactcaatatgtactcccacggtatagagatacaggagtttcatttgagataatgaggcgagcaaggagggaatgtaaagcacaaggagtgggtatgcttgcttggtctcatagggtcagggattttgaatacaaaacggtttataggagtgtgggatgaaaaagattttcaaggctgttgtaggtggaggcggcgggggtggaccatcaaaggaggaagccgccgcagcagaaagagcagcggcagaggctaacctgagggctcaacaagcagcacaggcgttgcaggaaaactttcgtgctgatctgagtacagacaatatcgcccagatcgctccgggtggtgaagctaatgctgcagggatggatgatgatttcaccccgcaaagaaaacgcaatagggtaggcggattgtctactcagttaggtatagggggtgacacatggctgtagat